European Patent Specification EP 3 766 503 B1, published July 24, 2024. Title: Application of microRNA-210 inhibitor in preparation of drugs for treating inflammatory skin diseases. Applicant: Second Xiang Ya Hospital of Central South University. The sequence listing filed with the application follows.

SEQUENCE LISTING (2 sequences)

SEQ ID NO: 1 - RNA, 22 nt, Homo sapiens
agucggcgacagugugcguguc

SEQ ID NO: 2 - RNA, 24 nt, Unknown
ucagccgcugugucacacgcacag